European Patent Application EP 4 644 555 A1, published November 5, 2025. Title: GALACTOSE-1-PHOSPHATE URIDYLTRANSFERASE MUTANT AND USE THEREOF IN PREPARATION OF L-LYSINE. Applicant: NINGXIA EPPEN BIOTECH CO., LTD. The sequence listing filed with the application follows.

SEQUENCE LISTING (24 sequences)

SEQ ID NO: 1 - DNA, 1287 bp, Corynebacterium glutamicum
  source 1..1287: mol_type = other DNA
atggctgacggcacgatcaaacagattcaccctttcacaggcaccgaagtgtggacggtccctgggcgtggaaatcgacctctgtcacatcccgcttctacgatcgtcgaactatctgcacacgatcacacctcttactgtgcattttgttccgacaatatgctctccactccgcctgagaaatcgcgcatcatcattgatagctccggcgactttgacatccttcccggagcattgcctggtgagctttcagaaaccactccggaatttcgacgagtccccaatctgtttgagattgtctcttttgactactggcaccagaattttggtttcgatatggattcagaaaccgccatgcgcatggcgcaatacttggcgattccagaaggtcgcgaacatgttttagccattgtgcgcacccgactttctgccgctggtgaagatcccgcgcacatgaccgatggcgagttgttagaaaaagctcccagctactttgctggtggtcatgacgtcatcatcggacgccgacactttgtcgatgacgcaaccaccagtgatcaattggcctcatctggaacactgaccgttaaagagcatgaggcgttcatccgcctgactgtcgatggcatcagggatttgtaccaccgcaaccgttacgcaccgtatgtagtggcgtttcaaaactggttgaaacccgccggcgcgtcttttgaccatcttcataaacagctcgtcgccattgatgaacgcggccgacttattgccgatgaactgcatcatctacgtggcaatcccaatatgtacaacgaacttgctgttgattacgccggataccacaacctgatcatcgcggaaaacgatcacgccgtggccttcgcaggtttcggtcaccgctaccccaccattgagatttactctaagtccgctattcctgaaccctggcttcaaagcgacgaggaaatccaagcgatgagcaacctcatccatgcatgccatgctgcaaccggcgcagatgtaccctgcaatgaggaatgggtacacaaaccaatcgatgttgatatgccaatgccctggcatgtgatgatcaaatggcgtgtttctaccctggcaggttttgaaggtggcaccaaggtgtatctcaatacgctgtctccacacaaggtccgagaccgtgtggtgaaagaaatgtaccgactacgcgatgaagaactcatcgcatctgatctgcgcatcgccatggaatgctccgttgaacgcaacagccttaaatacaatcccctcctataa

SEQ ID NO: 2 - protein, 428 aa, Corynebacterium glutamicum
MADGTIKQIHPFTGTEVWTVPGRGNRPLSHPASTIVELSAHDHTSYCAFCSDNMLSTPPEKSRIIIDSSGDFDILPGALPGELSETTPEFRRVPNLFEIVSFDYWHQNFGFDMDSETAMRMAQYLAIPEGREHVLAIVRTRLSAAGEDPAHMTDGELLEKAPSYFAGGHDVIIGRRHFVDDATTSDQLASSGTLTVKEHEAFIRLTVDGIRDLYHRNRYAPYVVAFQNWLKPAGASFDHLHKQLVAIDERGRLIADELHHLRGNPNMYNELAVDYAGYHNLIIAENDHAVAFAGFGHRYPTIEIYSKSAIPEPWLQSDEEIQAMSNLIHACHAATGADVPCNEEWVHKPIDVDMPMPWHVMIKWRVSTLAGFEGGTKVYLNTLSPHKVRDRVVKEMYRLRDEELIASDLRIAMECSVERNSLKYNPLL

SEQ ID NO: 3 - DNA, 1441 bp, synthetic construct
  source 1..1441: mol_type = other DNA
aattaagcttgcatgcctgcaggtcgactctagaggatcccaacaccacagtagacaatagccttggtgttatgactagcccccattctttttctgtcacccccattcgcaccatggctgacggcacgatcaaacagattcaccctttcacaggcaccgaagtgtggacggtccctgggcgtggaaatcgacctctgtcacatcccgcttctacgatcgtcgaactatctgcacacgatcacacctcttactgtgcattttgttccgacaatatgctctccactccgcctgagaaatcgcgcatcatcattgatagctccggcgactttgacatccttcccggagcattgcctggtgagctttcagaaaccactccggaatttcgacgagtccccaatctgtttgagattgtctcttttgactactggcaccagaattttggtttcgatatggattcagaaaccgccatgcgcatggcgcaatacttggcgattccagaaggtcgcgaacatgttttagccattgtgcgcacccgactttctgccgctggtgaagatcccgcgcacatgaccgatggcgagttgttagaaaaagctcccagctactttgctggtggtcatgacgtcatcatcggacgccgacactttgtcgatgacgcaaccaccagtgatcaattggcctcatctggaacactgaccgttaaagagcatgaggcgttcatccgcctgactgtcgatggcatcagggatttgtaccaccgcaaccgttacgcaccgtatgtagtggcgtttcaaaactggttgaaacccgccggcgcgtcttttgaccatcttcataaacagctcgtcgccattgatgaacgcggccgacttattgccgatgaactgcatcatctacgtggcaatcccaatatgtacaacgaacttgctgttgattacgccggataccacaacctgatcatcgcggaaaacgatcacgccgtggccttcgcaggtttcggtcaccgctaccccaccattgagatttactctaagtccgctattcctgaaccctggcttcaaagcgacgaggaaatccaagcgatgagcaacctcatccatgcatgccatgctgcaaccggcgcagatgtaccctgcaatgaggaatgggtacacaaaccaatcgatgttgatatgccaatgccctggcatgtgatgatcaaatggcgtgtttctaccctggcaggttttgaaggtggcaccaaggtgtatctcaatacgctgtctccacacaaggtccgagaccgtgtggtgaaagaaatgtaccgactacgcgatgaagaactcatcgcatctgatctgcgcatcgccatggaatgctccgttgaacgcaacagccttaaatacaatcccctcctataagaattcagcttggctgttttggcggatgagagaagattttc

SEQ ID NO: 4 - DNA, 1465 bp, synthetic construct
  source 1..1465: mol_type = other DNA
agcggataacaatttcacacaggaaacagaattaattaagcttgcatgcctgcaggtcgactctagaggatcccaacaccacagtagacaatagccttggtgttatgactagcccccattctttttctgtcacccccattcgcaccatggctgacggcacgatcaaacagattcaccctttcacaggcaccgaagtgtggacggtccctgggcgtggaaatcgacctctgtcacatcccgcttctacgatcgtcgaactatctgcacacgatcacacctcttactgtgcattttgttccgacaatatgctctccactccgcctgagaaatcgcgcatcatcattgatagctccggcgactttgacatccttcccggagcattgcctggtgagctttcagaaaccactccggaatttcgacgagtccccaatctgtttgagattgtctcttttgactactggcaccagaattttggtttcgatatggattcagaaaccgccatgcgcatggcgcaatacttggcgattccagaaggtcgcgaacatgttttagccattgtgcgcacccgactttctgccgctggtgaagatcccgcgcacatgaccgatggcgagttgttagaaaaagctcccagctactttgctggtggtcatgacgtcatcatcggacgccgacactttgtcgatgacgcaaccaccagtgatcaattggcctcatctggaacactgaccgttaaagagcatgaggcgttcatccgcctgactgtcgatggcatcagggatttgtaccaccgcaaccgttacgcaccgtatgtagtggcgtttcaaaactggttgaaacccgccggcgcgtcttttgaccatcttcataaacagctcgtcgccattgatgaacgcggccgacttattgccgatgaactgcatcatctacgtggcaatcccaatatgtacaacgaacttgctgttgattacgccggataccacaacctgatcatcgcggaaaacgatcacgccgtggccttcgcaggtttcggtcaccgctaccccaccattgagatttactctaagtccgctattcctgaaccctggcttcaaagcgacgaggaaatccaagcgatgagcaacctcatccatgcatgccatgctgcaaccggcgcagatgtaccctgcaatgaggaatgggtacacaaaccaatcgatgttgatatgccaatgccctggcatgtgatgatcaaatggcgtgtttctaccctggcaggttttgaaggtggcaccaaggtgtatctcaatacgctgtctccacacaaggtccgagaccgtgtggtgaaagaaatgtaccgactacgcgatgaagaactcatcgcatctgatctgcgcatcgccatggaatgctccgttgaacgcaacagccttaaatacaatcccctcctataagaattcagcttggctgttttggcggatgagag

SEQ ID NO: 5 - DNA, 1287 bp, synthetic construct
  source 1..1287: mol_type = other DNA
atggctgacggcacgatcaaacagattcaccctttcacaggcaccgaagtgtggacggtccctgggcgtggaaatcgacctctgtcacatcccgcttctacgatcgtcgaactatctgcacacgatcacacctcttactgtgcattttgttccgacaatatgctctccactccgcctgagaaatcgcgcatcatcattgatagctccggcgactttgacatccttcccggagcattgcctggtgagctttcagaaaccactccggaatttcgacgagtccccaatctgtttgagattgtctcttttgactactggcaccagaattttggtttcgatatggattcagaaaccgccatgcgcatggcgcaatacttggcgattccagaaggtcgcgaacatgttttagccattgtgcgcacccgactttctgccgctggtgaagatcccgcgcacatgaccgatggcgagttgttagaaaaagctcccagctactttgctggtggtcatgacgtcatcatcggacgccgacactttgtcgatgacgcaaccaccagtgatcaattggcctcatctggaacactgaccgttaaagagcatgaggcgttcatccgcctgactgtcgatggcatcagggatttgtaccaccgcaaccgttacgcaccgtatgtagtggcgtttcaaaactggttgaaacccgccggcgcgtcttttgaccatcttcataaacagctcgtcgccattgatgaacgcggccgacttattgccgatgaactgcatcatctacgtggcaatcccaatatgtacaacgaacttgctgttgattacgccggataccacaacctgatcatcgcggaaaacgatcacgccgtggccttcgcaggtttcggtcaccgctaccccaccattgagatttactctaagtccgctattcctgaaccctggcttcaaagcgacgaggaaatccaagcgatgagcaacctcatccatgcatgccatgctgcaaccggcgcagatgtaccctgcaatgaggaatgggtacacaaaccaatcgatgttgatatgccaatgccctggcatgtgatgatcaaatggcgtgtttctaccctggcaggttttgaaggtggcaccaaggtgtatctcaatacgctgtctccacacaaggtccgagaccgtgtggtgaaagaaatgtaccgactacgcgatgaagaactcatcgcatctgatctgcgcatcgccatgtaatgctccgttgaacgcaacagccttaaatacaatcccctcctataa

SEQ ID NO: 6 - protein, 427 aa, synthetic construct
MADGTIKQIHPFTGTEVWTVPGRGNRPLSHPASTIVELSAHDHTSYCAFCSDNMLSTPPEKSRIIIDSSGDFDILPGALPGELSETTPEFRRVPNLFEIVSFDYWHQNFGFDMDSETAMRMAQYLAIPEGREHVLAIVRTRLSAAGEDPAHMTDGELLEKAPSYFAGGHDVIIGRRHFVDDATTSDQLASSGTLTVKEHEAFIRLTVDGIRDLYHRNRYAPYVVAFQNWLKPAGASFDHLHKQLVAIDERGRLIADELHHLRGNPNMYNELAVDYAGYHNLIIAENDHAVAFAGFGHRYPTIEIYSKSAIPEPWLQSDEEIQAMSNLIHACHAATGADVPCNEEWVHKPIDVDMPMPWHVMIKWRVSTLAGFEGGTKVYLNTLSPHKVRDRVVKEMYRLRDEELIASDLRIAMCSVERNSLKYNPLL

SEQ ID NO: 7 - DNA, 1022 bp, synthetic construct
  source 1..1022: mol_type = other DNA
cagtgccaagcttgcatgcctgcaggtcgactctaggaactgcatcatctacgtggcaatcccaatatgtacaacgaacttgctgttgattacgccggataccacaacctgatcatcgcggaaaacgatcacgccgtggccttcgcaggtttcggtcaccgctaccccaccattgagatttactctaagtccgctattcctgaaccctggcttcaaagcgacgaggaaatccaagcgatgagcaacctcatccatgcatgccatgctgcaaccggcgcagatgtaccctgcaatgaggaatgggtacacaaaccaatcgatgttgatatgccaatgccctggcatgtgatgatcaaatggcgtgtttctaccctggcaggttttgaaggtggcaccaaggtgtatctcaatacgctgtctccacacaaggtccgagaccgtgtggtgaaagaaatgtaccgactacgcgatgaagaactcatcgcatctgatctgcgcatcgccatgtaatgctccgttgaacgcaacagccttaaatacaatcccctcctataagccaagagttttagtgtcgctgcgcaggtactctactatctaatccatgagccgcatttcagaacttctaaacaatcatggtgttgatctgtcgtggcaagaggccgcatatcaggatttccacgaacatcctgagctctccggcttcgaatcagagaccgcagatcgcattcagaaatacctcgagcgttttgattgtgaggtgattccaaatgttggcggttacggcattctggccgtgttccgaaatgggtcgacagatcctggtgcccctgttgcgttaatgcgcgcagatttcgatggccttcccgtcaaggaaatcaccggagttccgtttgcttccactcgtatgcgtccgcatgatggggcaaatgtccatgtcatgcacgcatgcggccacgatgtccacgtcaccgcgctgcttggtgcgggtaccgagctcgaattcgtaatcatggtcatagctg

SEQ ID NO: 8 - DNA, 1097 bp, synthetic construct
  source 1..1097: mol_type = other DNA
cagtgccaagcttgcatgcctgcaggtcgactctagcgtgatgcaggccgaaggatcgctcaagaatacgtagctcaaaactagcgaaggatctccacagtccatgggtagactgcaggaacttcataggcaagttcctgctccaggaggaaagcgtcctttggcaactctgctggcggggtgagcaaacgggcaaaaatcatggtcacttggttaacggagcctttaactccatcaacttcaatgaggtaacggttgaccgaggattcttccaagtctgcatcttcatgctcgtcgcggtaagtctggcgaagctgctcttccacagcttctgcgattttcgctgctggatcatggacaacaacgccatgatccatgaggcctttttcgatcaaaaggttggcgactacggtaaaacgtcccgctagtgcgatggaatctgtgtcggggactaaaacatcaaactgaatcttcggcataacaccacagtagacaatagccttggtgttatgactagcccccattctttttctgtcacccccattcgcaccgccaagagttttagtgtcgctgcgcaggtactctactatctaatccatgagccgcatttcagaacttctaaacaatcatggtgttgatctgtcgtggcaagaggccgcatatcaggatttccacgaacatcctgagctctccggcttcgaatcagagaccgcagatcgcattcagaaatacctcgagcgttttgattgtgaggtgattccaaatgttggcggttacggcattctggccgtgttccgaaatgggtcgacagatcctggtgcccctgttgcgttaatgcgcgcagatttcgatggccttcccgtcaaggaaatcaccggagttccgtttgcttccactcgtatgcgtccgcatgatggggcaaatgtccatgtcatgcacgcatgcggccacgatgtccacgtcaccgcgctgcttggtgcgtgtgccattttagatgagcgtcgcgatgcatgggaaggcacgttcatcgcgttgttccagccatcggaggaaaactccgggtaccgagctcgaattcgtaatcatggtcatagctg

SEQ ID NO: 9 - DNA, 66 bp, synthetic construct
  source 1..66: mol_type = other DNA
aattaagcttgcatgcctgcaggtcgactctagaggatcccaacaccacagtagacaatagccttg

SEQ ID NO: 10 - DNA, 66 bp, synthetic construct
  source 1..66: mol_type = other DNA
gaaaatcttctctcatccgccaaaacagccaagctgaattcttataggaggggattgtatttaagg

SEQ ID NO: 11 - DNA, 24 bp, synthetic construct
  source 1..24: mol_type = other DNA
agcggataacaatttcacacagga

SEQ ID NO: 12 - DNA, 19 bp, synthetic construct
  source 1..19: mol_type = other DNA
ctctcatccgccaaaacag

SEQ ID NO: 13 - DNA, 56 bp, synthetic construct
  source 1..56: mol_type = other DNA
cagtgccaagcttgcatgcctgcaggtcgactctaggaactgcatcatctacgtgg

SEQ ID NO: 14 - DNA, 30 bp, synthetic construct
  source 1..30: mol_type = other DNA
gcgttcaacggagcattacatggcgatgcg

SEQ ID NO: 15 - DNA, 31 bp, synthetic construct
  source 1..31: mol_type = other DNA
gatctgcgcatcgccatgtaatgctccgttg

SEQ ID NO: 16 - DNA, 58 bp, synthetic construct
  source 1..58: mol_type = other DNA
cagctatgaccatgattacgaattcgagctcggtacccgcaccaagcagcgcggtgac

SEQ ID NO: 17 - DNA, 18 bp, synthetic construct
  source 1..18: mol_type = other DNA
tgtaaaacgacggccagt

SEQ ID NO: 18 - DNA, 18 bp, synthetic construct
  source 1..18: mol_type = other DNA
caggaaacagctatgacc

SEQ ID NO: 19 - DNA, 21 bp, synthetic construct
  source 1..21: mol_type = other DNA
ctaccctggcaggttttgaag

SEQ ID NO: 20 - DNA, 20 bp, synthetic construct
  source 1..20: mol_type = other DNA
gaagttctgaaatgcggctc

SEQ ID NO: 21 - DNA, 57 bp, synthetic construct
  source 1..57: mol_type = other DNA
cagtgccaagcttgcatgcctgcaggtcgactctagcgtgatgcaggccgaaggatc

SEQ ID NO: 22 - DNA, 40 bp, synthetic construct
  source 1..40: mol_type = other DNA
gcgacactaaaactcttggcggtgcgaatgggggtgacag

SEQ ID NO: 23 - DNA, 40 bp, synthetic construct
  source 1..40: mol_type = other DNA
ctgtcacccccattcgcaccgccaagagttttagtgtcgc

SEQ ID NO: 24 - DNA, 59 bp, synthetic construct
  source 1..59: mol_type = other DNA
cagctatgaccatgattacgaattcgagctcggtacccggagttttcctccgatggctg